European Patent Specification EP 3 284 749 B1, published August 14, 2024. Title: A Set of Polypeptides Having Nuclease Activity or Nickase Activity, or Suppressing or Activating Expression of Target Gene, in a Photo-inducible or Chemically-inducible Manner. Applicant: The University of Tokyo. The sequence listing filed with the application follows.

SEQUENCE LISTING (28 sequences)

SEQ ID NO: 1 - protein, 186 aa, NEUROSPORA CRASSA
MSHTVNSSTMNPWEVEAYQQYHYDPRTAPTANPLFFHTLYAPGGYDIMGYLIQIMNRPNPQVELGPVDTSCALILCDLKQKDTPIVYASEAFLYMTGYSNAEVLGRNCRFLQSPDGMVKPKSTRKYVDSNTINTMRKAIDRNAEVQVEVVNFKKNGQRFVNFLTMIPVRDETGEYRYSMGFQCETE

SEQ ID NO: 2 - protein, 1368 aa, Streptococcus pyogenes [sequence omitted]

SEQ ID NO: 3 - protein, 939 aa, Artificial Sequence
  NLS-N713-GS-pMag-GS
MGTPKKKRKVGIHGVPAADKKYSIGLDIGTNSVGWAVITDEYKVPSKKFKVLGNTDRHSIKKNLIGALLFDSGETAEATRLKRTARRRYTRRKNRICYLQEIFSNEMAKVDDSFFHRLEESFLVEEDKKHERHPIFGNIVDEVAYHEKYPTIYHLRKKLVDSTDKADLRLIYLALAHMIKFRGHFLIEGDLNPDNSDVDKLFIQLVQTYNQLFEENPINASGVDAKAILSARLSKSRRLENLIAQLPGEKKNGLFGNLIALSLGLTPNFKSNFDLAEDAKLQLSKDTYDDDLDNLLAQIGDQYADLFLAAKNLSDAILLSDILRVNTEITKAPLSASMIKRYDEHHQDLTLLKALVRQQLPEKYKEIFFDQSKNGYAGYIDGGASQEEFYKFIKPILEKMDGTEELLVKLNREDLLRKQRTFDNGSIPHQIHLGELHAILRRQEDFYPFLKDNREKIEKILTFRIPYYVGPLARGNSRFAWMTRKSEETITPWNFEEVVDKGASAQSFIERMTNFDKNLPNEKVLPKHSLLYEYFTVYNELTKVKYVTEGMRKPAFLSGEQKKAIVDLLFKTNRKVTVKQLKEDYFKKIECFDSVEISGVEDRFNASLGTYHDLLKIIKDKDFLDNEENEDILEDIVLTLTLFEDREMIEERLKTYAHLFDDKVMKQLKRRRYTGWGRLSRKLINGIRDKQSGKTILDFLKSDGFANRNFMQLIHDDSLTFKEDIQKAQVEFGGSGSSGGSGHTLYAPGGYDIMGYLRQIRNRPNPQVELGPVDTSCALILCDLKQKDTPIVYASEAFLYMTGYSNAEVLGRNCRFLQSPDGMVKPKSTRKYVDSNTINTMRKAIDRNAEVQVEVVNFKKNGQRFVNFLTMIPVRDETGEYRYSMGFQCETEGGSGGSGGGSGSGSGGLESRGPFEGKPIPNPLLGLDSTRTGHHHHHH

SEQ ID NO: 4 - protein, 882 aa, Artificial Sequence
  GS-nMagHigh1-GS-C714-NLS
MGGSGSSGGSGGSGGSGHTLYAPGGYDIMGYLDQIGNRPNPQVELGPVDTSCALILCDLKQKDTPIVYASEAFLYMTGYSNAEVLGRNCRFLQSPDGMVKPKSTRKYVDSNTINTIRKAIDRNAEVQVEVVNFKKNGQRFVNFLTIIPVRDETGEYRYSMGFQCETEGGSGGSGGGSGSGSGGGTSGGGDSLHEHIANLAGSPAIKKGILQTVKVVDELVKVMGRHKPENIVIEMARENQTTQKGQKNSRERMKRIEEGIKELGSQILKEHPVENTQLQNEKLYLYYLQNGRDMYVDQELDINRLSDYDVDHIVPQSFLKDDSIDNKVLTRSDKNRGKSDNVPSEEVVKKMKNYWRQLLNAKLITQRKFDNLTKAERGGLSELDKAGFIKRQLVETRQITKHVAQILDSRMNTKYDENDKLIREVKVITLKSKLVSDFRKDFQFYKVREINNYHHAHDAYLNAVVGTALIKKYPKLESEFVYGDYKVYDVRKMIAKSEQEIGKATAKYFFYSNIMNFFKTEITLANGEIRKRPLIETNGETGEIVWDKGRDFATVRKVLSMPQVNIVKKTEVQTGGFSKESILPKRNSDKLIARKKDWDPKKYGGFDSPTVAYSVLVVAKVEKGKSKKLKSVKELLGITIMERSSFEKNPIDFLEAKGYKEVKKDLIIKLPKYSLFELENGRKRMLASAGELQKGNELALPSKYVNFLYLASHYEKLKGSPEDNEQKQLFVEQHKHYLDEIIEQISEFSKRVILADANLDKVLSAYNKHRDKPIREQAENIIHLFTLTNLGAPAAFKYFDTTIDRKRYTSTKEVLDATLIHQSITGLYETRIDLSQLGGDEFASPKKKRKVLESRGPFEGKPIPNPLLGLDSTRTGHHHHHH

SEQ ID NO: 5 - protein, 882 aa, Artificial Sequence
  GS-nMag-GS-C714-NLS
MGGSGSSGGSGGSGGSGHTLYAPGGYDIMGYLDQIGNRPNPQVELGPVDTSCALILCDLKQKDTPIVYASEAFLYMTGYSNAEVLGRNCRFLQSPDGMVKPKSTRKYVDSNTINTMRKAIDRNAEVQVEVVNFKKNGQRFVNFLTMIPVRDETGEYRYSMGFQCETEGGSGGSGGGSGSGSGGGTSGGGDSLHEHIANLAGSPAIKKGILQTVKVVDELVKVMGRHKPENIVIEMARENQTTQKGQKNSRERMKRIEEGIKELGSQILKEHPVENTQLQNEKLYLYYLQNGRDMYVDQELDINRLSDYDVDHIVPQSFLKDDSIDNKVLTRSDKNRGKSDNVPSEEVVKKMKNYWRQLLNAKLITQRKFDNLTKAERGGLSELDKAGFIKRQLVETRQITKHVAQILDSRMNTKYDENDKLIREVKVITLKSKLVSDFRKDFQFYKVREINNYHHAHDAYLNAVVGTALIKKYPKLESEFVYGDYKVYDVRKMIAKSEQEIGKATAKYFFYSNIMNFFKTEITLANGEIRKRPLIETNGETGEIVWDKGRDFATVRKVLSMPQVNIVKKTEVQTGGFSKESILPKRNSDKLIARKKDWDPKKYGGFDSPTVAYSVLVVAKVEKGKSKKLKSVKELLGITIMERSSFEKNPIDFLEAKGYKEVKKDLIIKLPKYSLFELENGRKRMLASAGELQKGNELALPSKYVNFLYLASHYEKLKGSPEDNEQKQLFVEQHKHYLDEIIEQISEFSKRVILADANLDKVLSAYNKHRDKPIREQAENIIHLFTLTNLGAPAAFKYFDTTIDRKRYTSTKEVLDATLIHQSITGLYETRIDLSQLGGDEFASPKKKRKVLESRGPFEGKPIPNPLLGLDSTRTGHHHHHH

SEQ ID NO: 6 - DNA, 1635 bp, Artificial Sequence
  StopFluc-1
atggaagatgccaaaaacattaagaagggcccagcgccattctacccactcgaagacgggaccgccggcgagcagctgcacaaagccatgaagcgctacgccctggtgcccggcaccatcgcctttaccgacgcacatatcgaggtggacattacctacgccgagtacttcgagatgagcgttcggctggcagaagctatgaagcgctatgggctgaatacaaaccatcggatcgtggtgtgcagcgagaatagcttgcagttcttcatgcccgtgttgggtgccctgttcatcggtgtggctgtggccccagctaacgacatctacaacgagcgcgagctgctgaacagcatgggcatcagccagcccaccgtcgtattcgtgagcaagaaagggctgcaaaagatcctcaacgtgcaaaagaagctaccgatcatacaaaagatcatcatcatggatagcaagaccgactaccagggcttccaaagcatgtacaccttcgtgacttcccatttgccacccggcttcaacgagtacgacttcgtgcccgagagcttcgaccgggacaaaaccatcgccctgatcatgaacagtagtggcagtaccggattgcccaagggcgtagccctaccgcaccgcaccgcttgtgtccgattcagtcatgcccgcgaccccatcttcggcaaccagatcatccccgacaccgctatcctcagcgtggtgccatttcaccacggcttcggcatgttcaccacgctgggctacttgatctgcggctttcgggtcgtgctcatgtaccgcttcgaggaggagctattcttgcgcagcttgcaagactataagattcaatctgccctgctggtgcccacactatttagcttcttcgctaagagcactctcatcgacaagtacgacctaagcaacttgcacgagatctaaagcggcggggcgccgctcagcaaggaggtaggtgaggccgtggccaaacgcttccacctaccaggcatccgccagggctacggcctgacagaaacaaccagcgccattctgatcacccccgaaggggacgacaagcctggcgcagtaggcaaggtggtgcccttcttcgaggctaaggtggtggacttggacaccggtaagacactgggtgtgaaccagcgcggcgagctgtgcgtccgtggccccatgatcatgagcggctacgttaacaaccccgaggctacaaacgctctcatcgacaaggacggctggctgcacagcggcgacatcgcctactgggacgaggacgagcacttcttcatcgtggaccggctgaagagcctgatcaaatacaagggctaccaggtagccccagccgaactggagagcatcctgctgcaacaccccaacatcttcgacgccggggtcgccggcctgcccgacgacgatgccggcgagctgcccgccgcagtcgtcgtgctggaacacggtaaaaccatgaccgagaaggagatcgtggactatgtggccagccaggttacaaccgccaagaagctgcgcggtggtgttgtgttcgtggacgaggtgcctaaaggactgaccggcaagttggacgcccgcaagatccgcgagattctcattaaggccaagaagtaa

SEQ ID NO: 7 - DNA, 1635 bp, Artificial Sequence
  StopFluc-2
atggaagatgccaaaaacattaagaagggcccagcgccattctacccactcgaagacgggaccgccggcgagcagctgcacaaagccatgaagcgctacgccctggtgcccggcaccatcgcctttaccgacgcacatatcgaggtggacattacctacgccgagtacttcgagatgagcgttcggctggcagaagctatgaagtaatatgggctgaatacaaaccatcggatcgtggtgtgcagcgagaatagcttgcagttcttcatgcccgtgttgggtgccctgttcatcggtgtggctgtggccccagctaacgacatctacaacgagcgcgagctgctgaacagcatgggcatcagccagcccaccgtcgtattcgtgagcaagaaagggctgcaaaagatcctcaacgtgcaaaagaagctaccgatcatacaaaagatcatcatcatggatagcaagaccgactaccagggcttccaaagcatgtacaccttcgtgacttcccatttgccacccggcttcaacgagtacgacttcgtgcccgagagcttcgaccgggacaaaaccatcgccctgatcatgaacagtagtggcagtaccggattgcccaagggcgtagccctaccgcaccgcaccgcttgtgtccgattcagtcatgcccgcgaccccatcttcggcaaccagatcatccccgacaccgctatcctcagcgtggtgccatttcaccacggcttcggcatgttcaccacgctgggctacttgatctgcggctttcgggtcgtgctcatgtaccgcttcgaggaggagctattcttgcgcagcttgcaagactataagattcaatctgccctgctggtgcccacactatttagcttcttcgctaagagcactctcatcgacaagtacgacctaagcaacttgcacgagatcgccagcggcggggcgccgctcagcaaggaggtaggtgaggccgtggccaaacgcttccacctaccaggcatccgccagggctacggcctgacagaaacaaccagcgccattctgatcacccccgaaggggacgacaagcctggcgcagtaggcaaggtggtgcccttcttcgaggctaaggtggtggacttggacaccggtaagacactgggtgtgaaccagcgcggcgagctgtgcgtccgtggccccatgatcatgagcggctacgttaacaaccccgaggctacaaacgctctcatcgacaaggacggctggctgcacagcggcgacatcgcctactgggacgaggacgagcacttcttcatcgtggaccggctgaagagcctgatcaaatacaagggctaccaggtagccccagccgaactggagagcatcctgctgcaacaccccaacatcttcgacgccggggtcgccggcctgcccgacgacgatgccggcgagctgcccgccgcagtcgtcgtgctggaacacggtaaaaccatgaccgagaaggagatcgtggactatgtggccagccaggttacaaccgccaagaagctgcgcggtggtgttgtgttcgtggacgaggtgcctaaaggactgaccggcaagttggacgcccgcaagatccgcgagattctcattaaggccaagaagtaa

SEQ ID NO: 8 - DNA, 1635 bp, Artificial Sequence
  StopFluc-3
atggaagatgccaaaaacattaagaagggcccagcgccattctacccactcgaagacgggaccgccggcgagcagctgcacaaagccatgaagcgctacgccctggtgcccggcaccatcgcctttaccgacgcacatatcgaggtggacattacctacgccgagtacttcgagatgagcgttcggctggcagaagctatgaagcgctatgggctgaatacaaaccatcggatcgtggtgtgcagcgagaatagcttgcagttcttcatgcccgtgttgggtgccctgttcatctaagtggctgtggccccagctaacgacatctacaacgagcgcgagctgctgaacagcatgggcatcagccagcccaccgtcgtattcgtgagcaagaaagggctgcaaaagatcctcaacgtgcaaaagaagctaccgatcatacaaaagatcatcatcatggatagcaagaccgactaccagggcttccaaagcatgtacaccttcgtgacttcccatttgccacccggcttcaacgagtacgacttcgtgcccgagagcttcgaccgggacaaaaccatcgccctgatcatgaacagtagtggcagtaccggattgcccaagggcgtagccctaccgcaccgcaccgcttgtgtccgattcagtcatgcccgcgaccccatcttcggcaaccagatcatccccgacaccgctatcctcagcgtggtgccatttcaccacggcttcggcatgttcaccacgctgggctacttgatctgcggctttcgggtcgtgctcatgtaccgcttcgaggaggagctattcttgcgcagcttgcaagactataagattcaatctgccctgctggtgcccacactatttagcttcttcgctaagagcactctcatcgacaagtacgacctaagcaacttgcacgagatctaaagcggcggggcgccgctcagcaaggaggtaggtgaggccgtggccaaacgcttccacctaccaggcatccgccagggctacggcctgacagaaacaaccagcgccattctgatcacccccgaaggggacgacaagcctggcgcagtaggcaaggtggtgcccttcttcgaggctaaggtggtggacttggacaccggtaagacactgggtgtgaaccagcgcggcgagctgtgcgtccgtggccccatgatcatgagcggctacgttaacaaccccgaggctacaaacgctctcatcgacaaggacggctggctgcacagcggcgacatcgcctactgggacgaggacgagcacttcttcatcgtggaccggctgaagagcctgatcaaatacaagggctaccaggtagccccagccgaactggagagcatcctgctgcaacaccccaacatcttcgacgccggggtcgccggcctgcccgacgacgatgccggcgagctgcccgccgcagtcgtcgtgctggaacacggtaaaaccatgaccgagaaggagatcgtggactatgtggccagccaggttacaaccgccaagaagctgcgcggtggtgttgtgttcgtggacgaggtgcctaaaggactgaccggcaagttggacgcccgcaagatccgcgagattctcattaaggccaagaagtaa

SEQ ID NO: 9 - protein, 914 aa, Artificial Sequence
  NES-dN713-GS-pMag-GS-NES
MGLPPLERLTLGSDKKYSIGLAIGTNSVGWAVITDEYKVPSKKFKVLGNTDRHSIKKNLIGALLFDSGETAEATRLKRTARRRYTRRKNRICYLQEIFSNEMAKVDDSFFHRLEESFLVEEDKKHERHPIFGNIVDEVAYHEKYPTIYHLRKKLVDSTDKADLRLIYLALAHMIKFRGHFLIEGDLNPDNSDVDKLFIQLVQTYNQLFEENPINASGVDAKAILSARLSKSRRLENLIAQLPGEKKNGLFGNLIALSLGLTPNFKSNFDLAEDAKLQLSKDTYDDDLDNLLAQIGDQYADLFLAAKNLSDAILLSDILRVNTEITKAPLSASMIKRYDEHHQDLTLLKALVRQQLPEKYKEIFFDQSKNGYAGYIDGGASQEEFYKFIKPILEKMDGTEELLVKLNREDLLRKQRTFDNGSIPHQIHLGELHAILRRQEDFYPFLKDNREKIEKILTFRIPYYVGPLARGNSRFAWMTRKSEETITPWNFEEVVDKGASAQSFIERMTNFDKNLPNEKVLPKHSLLYEYFTVYNELTKVKYVTEGMRKPAFLSGEQKKAIVDLLFKTNRKVTVKQLKEDYFKKIECFDSVEISGVEDRFNASLGTYHDLLKIIKDKDFLDNEENEDILEDIVLTLTLFEDREMIEERLKTYAHLFDDKVMKQLKRRRYTGWGRLSRKLINGIRDKQSGKTILDFLKSDGFANRNFMQLIHDDSLTFKEDIQKAQVGTGGSGSSGGSGHTLYAPGGYDIMGYLRQIRNRPNPQVELGPVDTSCALILCDLKQKDTPIVYASEAFLYMTGYSNAEVLGRNCRFLQSPDGMVKPKSTRKYVDSNTINTMRKAIDRNAEVQVEVVNFKKNGQRFVNFLTMIPVRDETGEYRYSMGFQCETEGGSGGSGGGSGSGSGGEFLPPLERLTL

SEQ ID NO: 10 - protein, 925 aa, Artificial Sequence
  GS-nMagHigh1-GS-dC714-GS-NLS-VP64
MGGSGSSGGSGGSGGSGHTLYAPGGYDIMGYLDQIGNRPNPQVELGPVDTSCALILCDLKQKDTPIVYASEAFLYMTGYSNAEVLGRNCRFLQSPDGMVKPKSTRKYVDSNTINTIRKAIDRNAEVQVEVVNFKKNGQRFVNFLTIIPVRDETGEYRYSMGFQCETEGGSGGSGGGSGSGSGGGTSGQGDSLHEHIANLAGSPAIKKGILQTVKVVDELVKVMGRHKPENIVIEMARENQTTQKGQKNSRERMKRIEEGIKELGSQILKEHPVENTQLQNEKLYLYYLQNGRDMYVDQELDINRLSDYDVDAIVPQSFLKDDSIDNKVLTRSDKNRGKSDNVPSEEVVKKMKNYWRQLLNAKLITQRKFDNLTKAERGGLSELDKAGFIKRQLVETRQITKHVAQILDSRMNTKYDENDKLIREVKVITLKSKLVSDFRKDFQFYKVREINNYHHAHDAYLNAVVGTALIKKYPKLESEFVYGDYKVYDVRKMIAKSEQEIGKATAKYFFYSNIMNFFKTEITLANGEIRKRPLIETNGETGEIVWDKGRDFATVRKVLSMPQVNIVKKTEVQTGGFSKESILPKRNSDKLIARKKDWDPKKYGGFDSPTVAYSVLVVAKVEKGKSKKLKSVKELLGITIMERSSFEKNPIDFLEAKGYKEVKKDLIIKLPKYSLFELENGRKRMLASAGELQKGNELALPSKYVNFLYLASHYEKLKGSPEDNEQKQLFVEQHKHYLDEIIEQISEFSKRVILADANLDKVLSAYNKHRDKPIREQAENIIHLFTLTNLGAPAAFKYFDTTIDRKRYTSTKEVLDATLIHQSITGLYETRIDLSQLGGDEFGGGGSGGGGSGGGGSGPKKKRKVAAAGSGRADALDDFDLDMLGSDALDDFDLDMLGSDALDDFDLDMLGSDALDDFDLDMLIN

SEQ ID NO: 11 - protein, 473 aa, Artificial Sequence
  NLS-GS-MS2-GS-NLS-p65-GS-HSF1
MGPKKKRKVGGSGMASNFTQFVLVDNGGTGDVTVAPSNFANGIAEWISSNSRSQAYKVTCSVRQSSAQNRKYTIKVEVPKGAWRSYLNMELTIPIFATNSDCELIVKAMQGLLKDGNPIPSAIAANSGIYAGGSGGSGGGSGSGSGSGPKKKRKVAAAGSPSGQISNQALALAPSSAPVLAQTMVPSSAMVPLAQPPAPAPVLTPGPPQSLSAPVPKSTQAGEGTLSEALLHLQFDADEDLGALLGNSTDPGVFTDLASVDNSEFQQLLNQGVSMSHSTAEPMLMEYPEAITRLVTGSQRPPDPAPTPLGTSGLPNGLSGDEDFSSIADMDFSALLSQISSSGQGGGGSGFSVDTSALLDLFSPSVTVPDMSLPDLDSSLASIQELLSPQEPPRPPEAENSSPDSGKQLVHYTAQPLFLLDPGSVDTGSNDLPVLFELGEGSYFSEGDGFAEDPTISLLTGSEPPKAKDPTVS

SEQ ID NO: 12 - DNA, 23 bp, Artificial Sequence
  StopFluc-1
  misc_feature (22)..(23): n is a, t, g or c
aacttgcacgagatctaaagcnn

SEQ ID NO: 13 - DNA, 23 bp, Artificial Sequence
  StopFluc-2
  misc_feature (22)..(23): n is a, t, g or c
gcagaagctatgaagtaatatnn

SEQ ID NO: 14 - DNA, 21 bp, Artificial Sequence
  sqRNA(StopFluc-1)
gaacttgcacgagatctaaag

SEQ ID NO: 15 - DNA, 20 bp, Artificial Sequence
  sgRNA(StopFluc-2)
gcagaagctatgaagtaata

SEQ ID NO: 16 - DNA, 20 bp, Artificial Sequence
  sgRNA(StopFluc-3)
gggtgccctgttcatctaag

SEQ ID NO: 17 - DNA, 38 bp, Homo sapiens
tatgacatcaattattatacatcggagccctgccaaaa

SEQ ID NO: 18 - DNA, 37 bp, Artificial Sequence
  1 bp deletion of human CCR5 locus
tatgacatcaattattatcatcggagccctgccaaaa

SEQ ID NO: 19 - DNA, 36 bp, Artificial Sequence
  2bp deletion of human CCR5 locus
tatgacatcaattattacatcggagccctgccaaaa

SEQ ID NO: 20 - DNA, 34 bp, Artificial Sequence
  4bp deletion of human CCR5 locus
tatgacatcaattattatcggagccctgccaaaa

SEQ ID NO: 21 - DNA, 28 bp, Artificial Sequence
  10bp deletion of human CCR5 locus
tatgacatcaattattatactgccaaaa

SEQ ID NO: 22 - DNA, 25 bp, Artificial Sequence
  13bp deletion of human CCR5 locus
tatgacatcaagagccctgccaaaa

SEQ ID NO: 23 - DNA, 24 bp, Artificial Sequence
  14bp deletion of human CCR5 locus
tatgacatcggagccctgccaaaa

SEQ ID NO: 24 - DNA, 38 bp, Homo sapiens
gaagggcctgagtccgagcagaagaagaagggctccca

SEQ ID NO: 25 - DNA, 38 bp, Homo sapiens
cttcccggactcaggctcgtcttcttcttcccgagggt

SEQ ID NO: 26 - DNA, 30 bp, Artificial Sequence
  ssODN 96 mer
tgagtccgagcagaagaagcttaagggctc

SEQ ID NO: 27 - DNA, 77 bp, Homo sapiens
agaaccggaggacaaagtacaaacggcagaagctggaggaggaagggcctgagtccgagcagaagaagaagggctcc

SEQ ID NO: 28 - DNA, 77 bp, Homo sapiens
tcttggcctcctgtttcatgtttgccgtcttcgacctcctccttcccggactcaggctcgtcttcttcttcccgagg